European Patent Specification EP 3 856 223 B1, published March 4, 2026. Title: Modified human erythropoietin. Applicant: Universidad Nacional del Litoral Consejo Nacional de Investigaciones Científicas y Técnicas (CONICET) Universidad Nacional de General San Martín. The sequence listing filed with the application follows.

SEQUENCE LISTING (26 sequences)

SEQ ID NO: 1 - DNA, 579 bp, DNA MUTEIN 15_17
atgggcgtgcacgaatgtcctgcttggctgtggctgctgctgtccctgctgtctctgcctctgggactgcctgtgctgggcgctcctcctagactgatctgcgactcccgggtgctggaaagaaacctgacggaagccaaagaggccgagaacatcaccaccggctgcgccgagcactgctccctgaacgagaatatcaccgtgcccgacaccaaagtgaacttctacgcctggaagcggatggaagtgggccagcaggctgtggaagtgtggcagggactggctctgctgagcgaggctgtgctgagaggacaggccctgctcgtgaactcctcccagccttgggaacccctgcagctgcacgtggacaaggctgtgtccggcctgagatccctgaccaccctgctgagagcactgggagcccagaaagaggccatctctccacctgacgccgcctctgctgctcctctgagaaccatcaccgccgacaccttcagaaagctgttccgggtgtactccaacttcctgcggggcaagctgaagctgtacaccggcgaggcttgccggaccggcgacaga

SEQ ID NO: 2 - protein, 193 aa, AA - MUTEIN 15_17
MGVHECPAWLWLLLSLLSLPLGLPVLGAPPRLICDSRVLERNLTEAKEAENITTGCAEHCSLNENITVPDTKVNFYAWKRMEVGQQAVEVWQGLALLSEAVLRGQALLVNSSQPWEPLQLHVDKAVSGLRSLTTLLRALGAQKEAISPPDAASAAPLRTITADTFRKLFRVYSNFLRGKLKLYTGEACRTGDR

SEQ ID NO: 3 - DNA, 579 bp, DNA MUTEIN 45_47
atgggcgtgcacgaatgtcctgcttggctgtggctgctgctgtccctgctgtctctgcctctgggactgcctgtgctgggcgctcctcctagactgatctgcgactcccgggtgctggaaagatacctgctggaagccaaagaggccgagaacatcaccaccggctgcgccgagcactgctccctgaacgagaatatcaccgtgcccgacaccaacgtgaccttctacgcctggaagcggatggaagtgggccagcaggctgtggaagtgtggcagggactggctctgctgagcgaggctgtgctgagaggacaggccctgctcgtgaactcctcccagccttgggaacccctgcagctgcacgtggacaaggctgtgtccggcctgagatccctgaccaccctgctgagagcactgggagcccagaaagaggccatctctccacctgacgccgcctctgctgctcctctgagaaccatcaccgccgacaccttcagaaagctgttccgggtgtactccaacttcctgcggggcaagctgaagctgtacaccggcgaggcttgccggaccggcgacaga

SEQ ID NO: 4 - protein, 193 aa, AA - MUTEIN 45_47
MGVHECPAWLWLLLSLLSLPLGLPVLGAPPRLICDSRVLERYLLEAKEAENITTGCAEHCSLNENITVPDTNVTFYAWKRMEVGQQAVEVWQGLALLSEAVLRGQALLVNSSQPWEPLQLHVDKAVSGLRSLTTLLRALGAQKEAISPPDAASAAPLRTITADTFRKLFRVYSNFLRGKLKLYTGEACRTGDR

SEQ ID NO: 5 - DNA, 579 bp, DNA MUTEIN 49
atgggcgtgcacgaatgtcctgcttggctgtggctgctgctgtccctgctgtctctgcctctgggactgcctgtgctgggcgctcctcctagactgatctgcgactcccgggtgctggaaagatacctgctggaagccaaagaggccgagaacatcaccaccggctgcgccgagcactgctccctgaacgagaatatcaccgtgcccgacaccaaagtgaacttcaccgcctggaagcggatggaagtgggccagcaggctgtggaagtgtggcagggactggctctgctgagcgaggctgtgctgagaggacaggccctgctcgtgaactcctcccagccttgggaacccctgcagctgcacgtggacaaggctgtgtccggcctgagatccctgaccaccctgctgagagcactgggagcccagaaagaggccatctctccacctgacgccgcctctgctgctcctctgagaaccatcaccgccgacaccttcagaaagctgttccgggtgtactccaacttcctgcggggcaagctgaagctgtacaccggcgaggcttgccggaccggcgacaga

SEQ ID NO: 6 - protein, 193 aa, AA - MUTEIN 49
MGVHECPAWLWLLLSLLSLPLGLPVLGAPPRLICDSRVLERYLLEAKEAENITTGCAEHCSLNENITVPDTKVNFTAWKRMEVGQQAVEVWQGLALLSEAVLRGQALLVNSSQPWEPLQLHVDKAVSGLRSLTTLLRALGAQKEAISPPDAASAAPLRTITADTFRKLFRVYSNFLRGKLKLYTGEACRTGDR

SEQ ID NO: 7 - DNA, 579 bp, DNA - MUTEIN 62_64
atgggcgtgcacgaatgtcctgcttggctgtggctgctgctgtccctgctgtctctgcctctgggactgcctgtgctgggcgctcctcctagactgatctgcgactcccgggtgctggaaagatacctgctggaagccaaagaggccgagaacatcaccaccggctgcgccgagcactgctccctgaacgagaatatcaccgtgcccgacaccaaagtgaacttctacgcctggaagcggatggaagtgggccagcaggctgtgaacgtgacgcagggactggctctgctgagcgaggctgtgctgagaggacaggccctgctcgtgaactcctcccagccttgggaacccctgcagctgcacgtggacaaggctgtgtccggcctgagatccctgaccaccctgctgagagcactgggagcccagaaagaggccatctctccacctgacgccgcctctgctgctcctctgagaaccatcaccgccgacaccttcagaaagctgttccgggtgtactccaacttcctgcggggcaagctgaagctgtacaccggcgaggcttgccggaccggcgacaga

SEQ ID NO: 8 - protein, 193 aa, AA - MUTEIN 62_64
MGVHECPAWLWLLLSLLSLPLGLPVLGAPPRLICDSRVLERYLLEAKEAENITTGCAEHCSLNENITVPDTKVNFYAWKRMEVGQQAVNVTQGLALLSEAVLRGQALLVNSSQPWEPLQLHVDKAVSGLRSLTTLLRALGAQKEAISPPDAASAAPLRTITADTFRKLFRVYSNFLRGKLKLYTGEACRTGDR

SEQ ID NO: 9 - DNA, 579 bp, DNA - MUTEIN  65_67
atgggcgtgcacgaatgtcctgcttggctgtggctgctgctgtccctgctgtctctgcctctgggactgcctgtgctgggcgctcctcctagactgatctgcgactcccgggtgctggaaagatacctgctggaagccaaagaggccgagaacatcaccaccggctgcgccgagcactgctccctgaacgagaatatcaccgtgcccgacaccaaagtgaacttctacgcctggaagcggatggaagtgggccagcaggctgtggaagtgtggaacggaacggctctgctgagcgaggctgtgctgagaggacaggccctgctcgtgaactcctcccagccttgggaacccctgcagctgcacgtggacaaggctgtgtccggcctgagatccctgaccaccctgctgagagcactgggagcccagaaagaggccatctctccacctgacgccgcctctgctgctcctctgagaaccatcaccgccgacaccttcagaaagctgttccgggtgtactccaacttcctgcggggcaagctgaagctgtacaccggcgaggcttgccggaccggcgacaga

SEQ ID NO: 10 - protein, 193 aa, AA - MUTEIN 65_67
MGVHECPAWLWLLLSLLSLPLGLPVLGAPPRLICDSRVLERYLLEAKEAENITTGCAEHCSLNENITVPDTKVNFYAWKRMEVGQQAVEVWNGTALLSEAVLRGQALLVNSSQPWEPLQLHVDKAVSGLRSLTTLLRALGAQKEAISPPDAASAAPLRTITADTFRKLFRVYSNFLRGKLKLYTGEACRTGDR

SEQ ID NO: 11 - DNA, 579 bp, DNA - MUTEIN 72_74
atgggcgtgcacgaatgtcctgcttggctgtggctgctgctgtccctgctgtctctgcctctgggactgcctgtgctgggcgctcctcctagactgatctgcgactcccgggtgctggaaagatacctgctggaagccaaagaggccgagaacatcaccaccggctgcgccgagcactgctccctgaacgagaatatcaccgtgcccgacaccaaagtgaacttctacgcctggaagcggatggaagtgggccagcaggctgtggaagtgtggcagggactggctctgctgagcaacgctacgctgagaggacaggccctgctcgtgaactcctcccagccttgggaacccctgcagctgcacgtggacaaggctgtgtccggcctgagatccctgaccaccctgctgagagcactgggagcccagaaagaggccatctctccacctgacgccgcctctgctgctcctctgagaaccatcaccgccgacaccttcagaaagctgttccgggtgtactccaacttcctgcggggcaagctgaagctgtacaccggcgaggcttgccggaccggcgacaga

SEQ ID NO: 12 - protein, 193 aa, AA - MUTEIN 72_74
MGVHECPAWLWLLLSLLSLPLGLPVLGAPPRLICDSRVLERYLLEAKEAENITTGCAEHCSLNENITVPDTKVNFYAWKRMEVGQQAVEVWQGLALLSNATLRGQALLVNSSQPWEPLQLHVDKAVSGLRSLTTLLRALGAQKEAISPPDAASAAPLRTITADTFRKLFRVYSNFLRGKLKLYTGEACRTGDR

SEQ ID NO: 13 - DNA, 579 bp, DNA - MUTEIN 76_78
atgggcgtgcacgaatgtcctgcttggctgtggctgctgctgtccctgctgtctctgcctctgggactgcctgtgctgggcgctcctcctagactgatctgcgactcccgggtgctggaaagatacctgctggaagccaaagaggccgagaacatcaccaccggctgcgccgagcactgctccctgaacgagaatatcaccgtgcccgacaccaaagtgaacttctacgcctggaagcggatggaagtgggccagcaggctgtggaagtgtggcagggactggctctgctgagcgaggctgtgctgaacggaacggccctgctcgtgaactcctcccagccttgggaacccctgcagctgcacgtggacaaggctgtgtccggcctgagatccctgaccaccctgctgagagcactgggagcccagaaagaggccatctctccacctgacgccgcctctgctgctcctctgagaaccatcaccgccgacaccttcagaaagctgttccgggtgtactccaacttcctgcggggcaagctgaagctgtacaccggcgaggcttgccggaccggcgacaga

SEQ ID NO: 14 - protein, 193 aa, AA- MUTEIN 76_78
MGVHECPAWLWLLLSLLSLPLGLPVLGAPPRLICDSRVLERYLLEAKEAENITTGCAEHCSLNENITVPDTKVNFYAWKRMEVGQQAVEVWQGLALLSEAVLNGTALLVNSSQPWEPLQLHVDKAVSGLRSLTTLLRALGAQKEAISPPDAASAAPLRTITADTFRKLFRVYSNFLRGKLKLYTGEACRTGDR

SEQ ID NO: 15 - DNA, 579 bp, DNA - MUTEIN 98_100
atgggcgtgcacgaatgtcctgcttggctgtggctgctgctgtccctgctgtctctgcctctgggactgcctgtgctgggcgctcctcctagactgatctgcgactcccgggtgctggaaagatacctgctggaagccaaagaggccgagaacatcaccaccggctgcgccgagcactgctccctgaacgagaatatcaccgtgcccgacaccaaagtgaacttctacgcctggaagcggatggaagtgggccagcaggctgtggaagtgtggcagggactggctctgctgagcgaggctgtgctgagaggacaggccctgctcgtgaactcctcccagccttgggaacccctgcagctgcacgtggacaagaatgtgaccggcctgagatccctgaccaccctgctgagagcactgggagcccagaaagaggccatctctccacctgacgccgcctctgctgctcctctgagaaccatcaccgccgacaccttcagaaagctgttccgggtgtactccaacttcctgcggggcaagctgaagctgtacaccggcgaggcttgccggaccggcgacaga

SEQ ID NO: 16 - protein, 193 aa, AA- MUTEIN 98_100
MGVHECPAWLWLLLSLLSLPLGLPVLGAPPRLICDSRVLERYLLEAKEAENITTGCAEHCSLNENITVPDTKVNFYAWKRMEVGQQAVEVWQGLALLSEAVLRGQALLVNSSQPWEPLQLHVDKNVTGLRSLTTLLRALGAQKEAISPPDAASAAPLRTITADTFRKLFRVYSNFLRGKLKLYTGEACRTGDR

SEQ ID NO: 17 - DNA, 579 bp, DNA - MUTEIN 104
atgggcgtgcacgaatgtcctgcttggctgtggctgctgctgtccctgctgtctctgcctctgggactgcctgtgctgggcgctcctcctagactgatctgcgactcccgggtgctggaaagatacctgctggaagccaaagaggccgagaacatcaccaccggctgcgccgagcactgctccctgaacgagaatatcaccgtgcccgacaccaaagtgaacttctacgcctggaagcggatggaagtgggccagcaggctgtggaagtgtggcagggactggctctgctgagcgaggctgtgctgagaggacaggccctgctcgtgaactcctcccagccttgggaacccctgcagctgcacgtggacaaggctgtgtccggcctgagaaacctgaccaccctgctgagagcactgggagcccagaaagaggccatctctccacctgacgccgcctctgctgctcctctgagaaccatcaccgccgacaccttcagaaagctgttccgggtgtactccaacttcctgcggggcaagctgaagctgtacaccggcgaggcttgccggaccggcgacaga

SEQ ID NO: 18 - protein, 193 aa, AA - MUTEIN 104
MGVHECPAWLWLLLSLLSLPLGLPVLGAPPRLICDSRVLERYLLEAKEAENITTGCAEHCSLNENITVPDTKVNFYAWKRMEVGQQAVEVWQGLALLSEAVLRGQALLVNSSQPWEPLQLHVDKAVSGLRNLTTLLRALGAQKEAISPPDAASAAPLRTITADTFRKLFRVYSNFLRGKLKLYTGEACRTGDR

SEQ ID NO: 19 - DNA, 579 bp, DNA - MUTEIN 106_108
atgggcgtgcacgaatgtcctgcttggctgtggctgctgctgtccctgctgtctctgcctctgggactgcctgtgctgggcgctcctcctagactgatctgcgactcccgggtgctggaaagatacctgctggaagccaaagaggccgagaacatcaccaccggctgcgccgagcactgctccctgaacgagaatatcaccgtgcccgacaccaaagtgaacttctacgcctggaagcggatggaagtgggccagcaggctgtggaagtgtggcagggactggctctgctgagcgaggctgtgctgagaggacaggccctgctcgtgaactcctcccagccttgggaacccctgcagctgcacgtggacaaggctgtgtccggcctgagatccctgaacaccacgctgagagcactgggagcccagaaagaggccatctctccacctgacgccgcctctgctgctcctctgagaaccatcaccgccgacaccttcagaaagctgttccgggtgtactccaacttcctgcggggcaagctgaagctgtacaccggcgaggcttgccggaccggcgacaga

SEQ ID NO: 20 - protein, 193 aa, AA - MUTEIN 106_108
MGVHECPAWLWLLLSLLSLPLGLPVLGAPPRLICDSRVLERYLLEAKEAENITTGCAEHCSLNENITVPDTKVNFYAWKRMEVGQQAVEVWQGLALLSEAVLRGQALLVNSSQPWEPLQLHVDKAVSGLRSLNTTLRALGAQKEAISPPDAASAAPLRTITADTFRKLFRVYSNFLRGKLKLYTGEACRTGDR

SEQ ID NO: 21 - DNA, 579 bp, DNA - MUTEIN 149
atgggcgtgcacgaatgtcctgcttggctgtggctgctgctgtccctgctgtctctgcctctgggactgcctgtgctgggcgctcctcctagactgatctgcgactcccgggtgctggaaagatacctgctggaagccaaagaggccgagaacatcaccaccggctgcgccgagcactgctccctgaacgagaatatcaccgtgcccgacaccaaagtgaacttctacgcctggaagcggatggaagtgggccagcaggctgtggaagtgtggcagggactggctctgctgagcgaggctgtgctgagaggacaggccctgctcgtgaactcctcccagccttgggaacccctgcagctgcacgtggacaaggctgtgtccggcctgagatccctgaccaccctgctgagagcactgggagcccagaaagaggccatctctccacctgacgccgcctctgctgctcctctgagaaccatcaccgccgacaccttcagaaagctgttccgggtgtactccaacttcacgcggggcaagctgaagctgtacaccggcgaggcttgccggaccggcgacaga

SEQ ID NO: 22 - protein, 193 aa, AA - MUTEIN 149
MGVHECPAWLWLLLSLLSLPLGLPVLGAPPRLICDSRVLERYLLEAKEAENITTGCAEHCSLNENITVPDTKVNFYAWKRMEVGQQAVEVWQGLALLSEAVLRGQALLVNSSQPWEPLQLHVDKAVSGLRSLTTLLRALGAQKEAISPPDAASAAPLRTITADTFRKLFRVYSNFTRGKLKLYTGEACRTGDR

SEQ ID NO: 23 - DNA, 579 bp, DNA - MUTEIN 151_153
atgggcgtgcacgaatgtcctgcttggctgtggctgctgctgtccctgctgtctctgcctctgggactgcctgtgctgggcgctcctcctagactgatctgcgactcccgggtgctggaaagatacctgctggaagccaaagaggccgagaacatcaccaccggctgcgccgagcactgctccctgaacgagaatatcaccgtgcccgacaccaaagtgaacttctacgcctggaagcggatggaagtgggccagcaggctgtggaagtgtggcagggactggctctgctgagcgaggctgtgctgagaggacaggccctgctcgtgaactcctcccagccttgggaacccctgcagctgcacgtggacaaggctgtgtccggcctgagatccctgaccaccctgctgagagcactgggagcccagaaagaggccatctctccacctgacgccgcctctgctgctcctctgagaaccatcaccgccgacaccttcagaaagctgttccgggtgtactccaacttcctgcggaacaagacgaagctgtacaccggcgaggcttgccggaccggcgacaga

SEQ ID NO: 24 - protein, 193 aa, AA - MUTEIN 151_153
MGVHECPAWLWLLLSLLSLPLGLPVLGAPPRLICDSRVLERYLLEAKEAENITTGCAEHCSLNENITVPDTKVNFYAWKRMEVGQQAVEVWQGLALLSEAVLRGQALLVNSSQPWEPLQLHVDKAVSGLRSLTTLLRALGAQKEAISPPDAASAAPLRTITADTFRKLFRVYSNFLRNKTKLYTGEACRTGDR

SEQ ID NO: 25 - DNA, 579 bp, DNA - hEPO
atgggcgtgcacgaatgtcctgcttggctgtggctgctgctgtccctgctgtctctgcctctgggactgcctgtgctgggcgctcctcctagactgatctgcgactcccgggtgctggaaagatacctgctggaagccaaagaggccgagaacatcaccaccggctgcgccgagcactgctccctgaacgagaatatcaccgtgcccgacaccaaagtgaacttctacgcctggaagcggatggaagtgggccagcaggctgtggaagtgtggcagggactggctctgctgagcgaggctgtgctgagaggacaggccctgctcgtgaactcctcccagccttgggaacccctgcagctgcacgtggacaaggctgtgtccggcctgagatccctgaccaccctgctgagagcactgggagcccagaaagaggccatctctccacctgacgccgcctctgctgctcctctgagaaccatcaccgccgacaccttcagaaagctgttccgggtgtactccaacttcctgcggggcaagctgaagctgtacaccggcgaggcttgccggaccggcgacaga

SEQ ID NO: 26 - protein, 193 aa, AA - hEPO
MGVHECPAWLWLLLSLLSLPLGLPVLGAPPRLICDSRVLERYLLEAKEAENITTGCAEHCSLNENITVPDTKVNFYAWKRMEVGQQAVEVWQGLALLSEAVLRGQALLVNSSQPWEPLQLHVDKAVSGLRSLTTLLRALGAQKEAISPPDAASAAPLRTITADTFRKLFRVYSNFLRGKLKLYTGEACRTGDR